European Patent Application EP 4 806 913 A1, published September 16, 2026. Title: EphA2를 타겟하는 개선된 특성을 갖는 친수성 모노바디 및 이를 포함하는 다중특이적 키메라 항원 수용체 및 조작된 면역세포. Applicant: 주식회사 박셀바이오. Application KR. The sequence listing filed with the application follows.

SEQUENCE LISTING (58 sequences)

SEQ ID NO: 1 - protein, 63 aa, synthetic construct
ATGGCCCTGCCTGTGACAGCTTTGCTGCTGCCTCTGGCTCTGCTGCTGCATGCTGCTAGACCT

SEQ ID NO: 2 - protein, 291 aa, synthetic construct
AGCAGCGACAGCCCCAGAAATCTGGAAGTGACCAACGCCACACCTAACAGCCTGACCATCAGCTGGTACTACCCCTTCTGCGCCTTCTACTACCGGATCACCTATGGCGAGACAGGCGGCAACAGCCCTAGCCAAGAGTTCACCGTGCCTAGACCTAGCGACACCGCCACAATCTCTGGCCTGAAGCCAGGCCAGGACTACACCATCACAGTGTACGCCGTGACCTGCCTGGGCAGCTACAGCAGACCCATCAGCATCAACTACCGGACCGAGATCGACAAGCCCAGCCAA

SEQ ID NO: 3 - protein, 207 aa, synthetic construct
ACCACCACACCAGCTCCACGGCCTCCAACACCAGCACCTACAATTGCCTCTCAGCCCCTGTCTCTGAGGCCAGAAGCTTGTAGACCTGCTGCAGGCGGAGCCGTGCATACCAGAGGACTGGATTTCGCCTGCGACATCTACATTTGGGCCCCTCTGGCTGGAACATGTGGCGTCCTGCTGCTGTCTCTCGTGATCACCCTGTACTGC

SEQ ID NO: 4 - protein, 123 aa, synthetic construct
AGAAGCAAGAGAAGCCGGCTGCTGCACAGCGACTACATGAACATGACCCCTAGACGGCCCGGACCTACCAGAAAGCACTACCAGCCTTACGCTCCTCCTCGGGACTTTGCCGCCTATAGATCC

SEQ ID NO: 5 - protein, 126 aa, synthetic construct
AAGCGGGGCAGAAAGAAGCTGCTGTACATCTTCAAGCAGCCCTTCATGCGGCCCGTGCAGACCACACAAGAGGAAGATGGCTGCTCCTGCAGATTCCCCGAGGAAGAAGAAGGCGGCTGCGAGCTG

SEQ ID NO: 6 - protein, 339 aa, synthetic construct
AGAGTGAAGTTCTCTAGATCTGCCGACGCTCCTGCCTACCAGCAGGGACAGAATCAGCTGTACAACGAGCTGAATCTGGGGCGCAGAGAAGAGTACGACGTGCTGGATAAGAGAAGAGGCAGAGATCCCGAGATGGGCGGCAAGCCCCAGAGAAGAAAGAATCCCCAAGAGGGCCTGTATAATGAGCTGCAGAAAGACAAGATGGCCGAGGCCTACAGCGAGATCGGAATGAAGGGCGAACGCAGAAGAGGAAAGGGCCACGACGGACTGTATCAGGGCCTGAGCACAGCCACCAAGGATACCTATGATGCCCTGCACATGCAGGCCCTGCCACCTAGG

SEQ ID NO: 7 - protein, 21 aa, synthetic construct
MALPVTALLLPLALLLHAARP

SEQ ID NO: 8 - protein, 97 aa, synthetic construct
SSDSPRNLEVTNATPNSLTISWYYPFCAFYYRITYGETGGNSPSQEFTVPRPSDTATISGLKPGQDYTITVYAVTCLGSYSRPISINYRTEIDKPSQ

SEQ ID NO: 9 - protein, 69 aa, synthetic construct
TTTPAPRPPTPAPTIASQPLSLRPEACRPAAGGAVHTRGLDFACDIYIWAPLAGTCGVLLLSLVITLYC

SEQ ID NO: 10 - protein, 41 aa, synthetic construct
RSKRSRLLHSDYMNMTPRRPGPTRKHYQPYAPPRDFAAYRS

SEQ ID NO: 11 - protein, 42 aa, synthetic construct
KRGRKKLLYIFKQPFMRPVQTTQEEDGCSCRFPEEEEGGCEL

SEQ ID NO: 12 - protein, 113 aa, synthetic construct
RVKFSRSADAPAYQQGQNQLYNELNLGRREEYDVLDKRRGRDPEMGGKPQRRKNPQEGLYNELQKDKMAEAYSEIGMKGERRRGKGHDGLYQGLSTATKDTYDALHMQALPPR

SEQ ID NO: 13 - protein, 17 aa, synthetic construct
ACCACCACACCAGCTCC

SEQ ID NO: 14 - protein, 18 aa, synthetic construct
AGGTCTAGCAGCATGCAG

SEQ ID NO: 15 - protein, 30 aa, synthetic construct
CATGCTGCTAGACCTAGCAGCGACAGCCCC

SEQ ID NO: 16 - protein, 33 aa, synthetic construct
AGCTGGTGTGGTGGTTTGGCTGGGCTTGTCGAT

SEQ ID NO: 17 - protein, 63 aa, synthetic construct; identical to SEQ ID NO: 1

SEQ ID NO: 18 - protein, 765 aa, synthetic construct
CAGATGCAGCTGGTGCAGTCTGGGGCTGAGGTGAAGAAGCCTGGGTCCTCGGTGAAGGTCTCCTGCAAGGCTTCTGGAGGCACCTTCAGCAGCTATGCTATCAGCTGGGTGCGACAGGCCCCTGGACAAGGGCTTGAGTGGATGGGAAGGATCATCCCTATCCTTGGTATAGCAAACTACGCACAGAAGTTCCAGGGCAGAGTCACGATTACCGCGGACAAATCCACGAGCACAGCCTACATGGAGCTGAGCAGCCTGAGATCTGAGGACACGGCCGTGTATTACTGTGCGAAACCGAGAGATGGCTACAATTTGGTTGCTTTTGATATCTGGGGCCAAGGGACGATGGTCACCGTCTCCTCAGGCCTCGGGGGCCTCGGAGGAGGAGGTAGTGGCGGAGGAGGCTCCGGTGGATCCAGCGGTGTGGGTTCCCAGCTCGTGCTGACTCAGCCGCCCTCAGTGTCTGGGGCCCCAGGGCAGAGGGTCACCATCTCCTGCACTGGGAGCAGCTCCAACATCGGGGCAGGTTATGATGTACACTGGTATCAGCAACTTCCAGGAGCAGCCCCCAAACTCCTCATCTATGGCGACATCAATCGGCCCTCAGGGGTCCCTGACCGATTCTCTGGCTCCAAGTCTGGCATCTCAGCCTCCCTGGCTATCACTGGGCTCCAGGCTGAGGACGAGGCTGATTATTACTGCCAGTCCTATGACAGCAGCCTGAGTGGGGGGGTGTTCGGCGGAGGGACCAAGCTGACCGTCCTA

SEQ ID NO: 19 - protein, 45 aa, synthetic construct
GGAGGCGGAGGTTCTGGCGGCGGAGGAAGTGGTGGCGGAGGCTCT

SEQ ID NO: 20 - protein, 291 aa, synthetic construct; identical to SEQ ID NO: 2

SEQ ID NO: 21 - protein, 24 aa, synthetic construct
GACTACAAGGACGACGATGACAAG

SEQ ID NO: 22 - protein, 207 aa, synthetic construct; identical to SEQ ID NO: 3

SEQ ID NO: 23 - protein, 123 aa, synthetic construct; identical to SEQ ID NO: 4

SEQ ID NO: 24 - protein, 126 aa, synthetic construct; identical to SEQ ID NO: 5

SEQ ID NO: 25 - protein, 339 aa, synthetic construct; identical to SEQ ID NO: 6

SEQ ID NO: 26 - protein, 21 aa, synthetic construct
MALPVTALLLPLALLLHAARP

SEQ ID NO: 27 - protein, 255 aa, synthetic construct
QMQLVQSGAEVKKPGSSVKVSCKASGGTFSSYAISWVRQAPGQGLEWMGRIIPILGIANYAQKFQGRVTITADKSTSTAYMELSSLRSEDTAVYYCAKPRDGYNLVAFDIWGQGTMVTVSSGLGGLGGGGSGGGGSGGSSGVGSQLVLTQPPSVSGAPGQRVTISCTGSSSNIGAGYDVHWYQQLPGAAPKLLIYGDINRPSGVPDRFSGSKSGISASLAITGLQAEDEADYYCQSYDSSLSGGVFGGGTKLTVL

SEQ ID NO: 28 - protein, 15 aa, synthetic construct
GGGGSGGGGSGGGGS

SEQ ID NO: 29 - protein, 97 aa, synthetic construct; identical to SEQ ID NO: 8

SEQ ID NO: 30 - protein, 8 aa, synthetic construct
DYKDDDDK

SEQ ID NO: 31 - protein, 69 aa, synthetic construct; identical to SEQ ID NO: 9

SEQ ID NO: 32 - protein, 41 aa, synthetic construct; identical to SEQ ID NO: 10

SEQ ID NO: 33 - protein, 42 aa, synthetic construct; identical to SEQ ID NO: 11

SEQ ID NO: 34 - protein, 113 aa, synthetic construct; identical to SEQ ID NO: 12

SEQ ID NO: 35 - protein, 17 aa, synthetic construct
ACCACCACACCAGCTCC

SEQ ID NO: 36 - protein, 18 aa, synthetic construct
AGGTCTAGCAGCATGCAG

SEQ ID NO: 37 - protein, 36 aa, synthetic construct
CTGCATGCTGCTAGACCTCAGATGCAGCTGGTGCAG

SEQ ID NO: 38 - protein, 65 aa, synthetic construct
AGAGCCTCCGCCACCACTTCCTCCGCCGCCAGAACCTCCGCCTCCTAGGACGGTCAGCTTGGTCC

SEQ ID NO: 39 - protein, 31 aa, synthetic construct
GGTGGCGGAGGCTCTAGCAGCGACAGCCCCA

SEQ ID NO: 40 - protein, 58 aa, synthetic construct
AGCTGGTGTGGTGGTCTTGTCATCGTCGTCCTTGTAGTCTTGGCTGGGCTTGTCGATC

SEQ ID NO: 41 - protein, 30 aa, synthetic construct; identical to SEQ ID NO: 15

SEQ ID NO: 42 - protein, 66 aa, synthetic construct
AGAGCCTCCGCCACCACTTCCTCCGCCGCCAGAACCTCCGCCTCCTTGGCTGGGCTTGTCGATCTC

SEQ ID NO: 43 - protein, 33 aa, synthetic construct
GGTGGCGGAGGCTCTCAGATGCAGCTGGTGCAG

SEQ ID NO: 44 - protein, 59 aa, synthetic construct
AGCTGGTGTGGTGGTCTTGTCATCGTCGTCCTTGTAGTCTAGGACGGTCAGCTTGGTCC

SEQ ID NO: 45 - protein, 270 aa, synthetic construct
GTTTCTGATGTTCCGAGGGACCTGGAAGTTGTTGCTGCGACCCCCACCAGCCTACTGATCAGCTGGTATTATCCGTTTTGTGCGTTTTATTACAGGATCACTTACGGAGAAACAGGAGGAAATAGCCCTGTCCAGGAGTTCACTGTGCCTCGTCCGTCTGACACTGCTACCATCAGCGGCCTTAAACCTGGAGTTGATTATACCATCACTGTGTATGCTGTCACGTGTCTGGGCTCGTATTCTCGCCCAATTTCCATTAATTACCGAACA

SEQ ID NO: 46 - protein, 90 aa, synthetic construct
VSDVPRDLEVVAATPTSLLISWYYPFCAFYYRITYGETGGNSPVQEFTVPRPSDTATISGLKPGVDYTITVYAVTCLGSYSRPISINYRT

SEQ ID NO: 47 - protein, 1857 aa, synthetic construct
ATGGCCCTGCCTGTGACAGCTTTGCTGCTGCCTCTGGCTCTGCTGCTGCATGCTGCTAGACCTCAGATGCAGCTGGTGCAGTCTGGGGCTGAGGTGAAGAAGCCTGGGTCCTCGGTGAAGGTCTCCTGCAAGGCTTCTGGAGGCACCTTCAGCAGCTATGCTATCAGCTGGGTGCGACAGGCCCCTGGACAAGGGCTTGAGTGGATGGGAAGGATCATCCCTATCCTTGGTATAGCAAACTACGCACAGAAGTTCCAGGGCAGAGTCACGATTACCGCGGACAAATCCACGAGCACAGCCTACATGGAGCTGAGCAGCCTGAGATCTGAGGACACGGCCGTGTATTACTGTGCGAAACCGAGAGATGGCTACAATTTGGTTGCTTTTGATATCTGGGGCCAAGGGACGATGGTCACCGTCTCCTCAGGCCTCGGGGGCCTCGGAGGAGGAGGTAGTGGCGGAGGAGGCTCCGGTGGATCCAGCGGTGTGGGTTCCCAGCTCGTGCTGACTCAGCCGCCCTCAGTGTCTGGGGCCCCAGGGCAGAGGGTCACCATCTCCTGCACTGGGAGCAGCTCCAACATCGGGGCAGGTTATGATGTACACTGGTATCAGCAACTTCCAGGAGCAGCCCCCAAACTCCTCATCTATGGCGACATCAATCGGCCCTCAGGGGTCCCTGACCGATTCTCTGGCTCCAAGTCTGGCATCTCAGCCTCCCTGGCTATCACTGGGCTCCAGGCTGAGGACGAGGCTGATTATTACTGCCAGTCCTATGACAGCAGCCTGAGTGGGGGGGTGTTCGGCGGAGGGACCAAGCTGACCGTCCTAGGAGGCGGAGGTTCTGGCGGCGGAGGAAGTGGTGGCGGAGGCTCTAGCAGCGACAGCCCCAGAAATCTGGAAGTGACCAACGCCACACCTAACAGCCTGACCATCAGCTGGTACTACCCCTTCTGCGCCTTCTACTACCGGATCACCTATGGCGAGACAGGCGGCAACAGCCCTAGCCAAGAGTTCACCGTGCCTAGACCTAGCGACACCGCCACAATCTCTGGCCTGAAGCCAGGCCAGGACTACACCATCACAGTGTACGCCGTGACCTGCCTGGGCAGCTACAGCAGACCCATCAGCATCAACTACCGGACCGAGATCGACAAGCCCAGCCAAGACTACAAGGACGACGATGACAAGACCACCACACCAGCTCCACGGCCTCCAACACCAGCACCTACAATTGCCTCTCAGCCCCTGTCTCTGAGGCCAGAAGCTTGTAGACCTGCTGCAGGCGGAGCCGTGCATACCAGAGGACTGGATTTCGCCTGCGACATCTACATTTGGGCCCCTCTGGCTGGAACATGTGGCGTCCTGCTGCTGTCTCTCGTGATCACCCTGTACTGCAGAAGCAAGAGAAGCCGGCTGCTGCACAGCGACTACATGAACATGACCCCTAGACGGCCCGGACCTACCAGAAAGCACTACCAGCCTTACGCTCCTCCTCGGGACTTTGCCGCCTATAGATCCAGAGTGAAGTTCTCTAGATCTGCCGACGCTCCTGCCTACCAGCAGGGACAGAATCAGCTGTACAACGAGCTGAATCTGGGGCGCAGAGAAGAGTACGACGTGCTGGATAAGAGAAGAGGCAGAGATCCCGAGATGGGCGGCAAGCCCCAGAGAAGAAAGAATCCCCAAGAGGGCCTGTATAATGAGCTGCAGAAAGACAAGATGGCCGAGGCCTACAGCGAGATCGGAATGAAGGGCGAACGCAGAAGAGGAAAGGGCCACGACGGACTGTATCAGGGCCTGAGCACAGCCACCAAGGATACCTATGATGCCCTGCACATGCAGGCCCTGCCACCTAGG

SEQ ID NO: 48 - protein, 1857 aa, synthetic construct
ATGGCCCTGCCTGTGACAGCTTTGCTGCTGCCTCTGGCTCTGCTGCTGCATGCTGCTAGACCTAGCAGCGACAGCCCCAGAAATCTGGAAGTGACCAACGCCACACCTAACAGCCTGACCATCAGCTGGTACTACCCCTTCTGCGCCTTCTACTACCGGATCACCTATGGCGAGACAGGCGGCAACAGCCCTAGCCAAGAGTTCACCGTGCCTAGACCTAGCGACACCGCCACAATCTCTGGCCTGAAGCCAGGCCAGGACTACACCATCACAGTGTACGCCGTGACCTGCCTGGGCAGCTACAGCAGACCCATCAGCATCAACTACCGGACCGAGATCGACAAGCCCAGCCAAGGAGGCGGAGGTTCTGGCGGCGGAGGAAGTGGTGGCGGAGGCTCTCAGATGCAGCTGGTGCAGTCTGGGGCTGAGGTGAAGAAGCCTGGGTCCTCGGTGAAGGTCTCCTGCAAGGCTTCTGGAGGCACCTTCAGCAGCTATGCTATCAGCTGGGTGCGACAGGCCCCTGGACAAGGGCTTGAGTGGATGGGAAGGATCATCCCTATCCTTGGTATAGCAAACTACGCACAGAAGTTCCAGGGCAGAGTCACGATTACCGCGGACAAATCCACGAGCACAGCCTACATGGAGCTGAGCAGCCTGAGATCTGAGGACACGGCCGTGTATTACTGTGCGAAACCGAGAGATGGCTACAATTTGGTTGCTTTTGATATCTGGGGCCAAGGGACGATGGTCACCGTCTCCTCAGGCCTCGGGGGCCTCGGAGGAGGAGGTAGTGGCGGAGGAGGCTCCGGTGGATCCAGCGGTGTGGGTTCCCAGCTCGTGCTGACTCAGCCGCCCTCAGTGTCTGGGGCCCCAGGGCAGAGGGTCACCATCTCCTGCACTGGGAGCAGCTCCAACATCGGGGCAGGTTATGATGTACACTGGTATCAGCAACTTCCAGGAGCAGCCCCCAAACTCCTCATCTATGGCGACATCAATCGGCCCTCAGGGGTCCCTGACCGATTCTCTGGCTCCAAGTCTGGCATCTCAGCCTCCCTGGCTATCACTGGGCTCCAGGCTGAGGACGAGGCTGATTATTACTGCCAGTCCTATGACAGCAGCCTGAGTGGGGGGGTGTTCGGCGGAGGGACCAAGCTGACCGTCCTAGACTACAAGGACGACGATGACAAGACCACCACACCAGCTCCACGGCCTCCAACACCAGCACCTACAATTGCCTCTCAGCCCCTGTCTCTGAGGCCAGAAGCTTGTAGACCTGCTGCAGGCGGAGCCGTGCATACCAGAGGACTGGATTTCGCCTGCGACATCTACATTTGGGCCCCTCTGGCTGGAACATGTGGCGTCCTGCTGCTGTCTCTCGTGATCACCCTGTACTGCAGAAGCAAGAGAAGCCGGCTGCTGCACAGCGACTACATGAACATGACCCCTAGACGGCCCGGACCTACCAGAAAGCACTACCAGCCTTACGCTCCTCCTCGGGACTTTGCCGCCTATAGATCCAGAGTGAAGTTCTCTAGATCTGCCGACGCTCCTGCCTACCAGCAGGGACAGAATCAGCTGTACAACGAGCTGAATCTGGGGCGCAGAGAAGAGTACGACGTGCTGGATAAGAGAAGAGGCAGAGATCCCGAGATGGGCGGCAAGCCCCAGAGAAGAAAGAATCCCCAAGAGGGCCTGTATAATGAGCTGCAGAAAGACAAGATGGCCGAGGCCTACAGCGAGATCGGAATGAAGGGCGAACGCAGAAGAGGAAAGGGCCACGACGGACTGTATCAGGGCCTGAGCACAGCCACCAAGGATACCTATGATGCCCTGCACATGCAGGCCCTGCCACCTAGG

SEQ ID NO: 49 - protein, 1023 aa, synthetic construct
ATGGCCCTGCCTGTGACAGCTTTGCTGCTGCCTCTGGCTCTGCTGCTGCATGCTGCTAGACCTAGCAGCGACAGCCCCAGAAATCTGGAAGTGACCAACGCCACACCTAACAGCCTGACCATCAGCTGGTACTACCCCTTCTGCGCCTTCTACTACCGGATCACCTATGGCGAGACAGGCGGCAACAGCCCTAGCCAAGAGTTCACCGTGCCTAGACCTAGCGACACCGCCACAATCTCTGGCCTGAAGCCAGGCCAGGACTACACCATCACAGTGTACGCCGTGACCTGCCTGGGCAGCTACAGCAGACCCATCAGCATCAACTACCGGACCGAGATCGACAAGCCCAGCCAAACCACCACACCAGCTCCACGGCCTCCAACACCAGCACCTACAATTGCCTCTCAGCCCCTGTCTCTGAGGCCAGAAGCTTGTAGACCTGCTGCAGGCGGAGCCGTGCATACCAGAGGACTGGATTTCGCCTGCGACATCTACATTTGGGCCCCTCTGGCTGGAACATGTGGCGTCCTGCTGCTGTCTCTCGTGATCACCCTGTACTGCAGAAGCAAGAGAAGCCGGCTGCTGCACAGCGACTACATGAACATGACCCCTAGACGGCCCGGACCTACCAGAAAGCACTACCAGCCTTACGCTCCTCCTCGGGACTTTGCCGCCTATAGATCCAGAGTGAAGTTCTCTAGATCTGCCGACGCTCCTGCCTACCAGCAGGGACAGAATCAGCTGTACAACGAGCTGAATCTGGGGCGCAGAGAAGAGTACGACGTGCTGGATAAGAGAAGAGGCAGAGATCCCGAGATGGGCGGCAAGCCCCAGAGAAGAAAGAATCCCCAAGAGGGCCTGTATAATGAGCTGCAGAAAGACAAGATGGCCGAGGCCTACAGCGAGATCGGAATGAAGGGCGAACGCAGAAGAGGAAAGGGCCACGACGGACTGTATCAGGGCCTGAGCACAGCCACCAAGGATACCTATGATGCCCTGCACATGCAGGCCCTGCCACCTAGG

SEQ ID NO: 50 - protein, 1026 aa, synthetic construct
ATGGCCCTGCCTGTGACAGCTTTGCTGCTGCCTCTGGCTCTGCTGCTGCATGCTGCTAGACCTAGCAGCGACAGCCCCAGAAATCTGGAAGTGACCAACGCCACACCTAACAGCCTGACCATCAGCTGGTACTACCCCTTCTGCGCCTTCTACTACCGGATCACCTATGGCGAGACAGGCGGCAACAGCCCTAGCCAAGAGTTCACCGTGCCTAGACCTAGCGACACCGCCACAATCTCTGGCCTGAAGCCAGGCCAGGACTACACCATCACAGTGTACGCCGTGACCTGCCTGGGCAGCTACAGCAGACCCATCAGCATCAACTACCGGACCGAGATCGACAAGCCCAGCCAAACCACCACACCAGCTCCACGGCCTCCAACACCAGCACCTACAATTGCCTCTCAGCCCCTGTCTCTGAGGCCAGAAGCTTGTAGACCTGCTGCAGGCGGAGCCGTGCATACCAGAGGACTGGATTTCGCCTGCGACATCTACATTTGGGCCCCTCTGGCTGGAACATGTGGCGTCCTGCTGCTGTCTCTCGTGATCACCCTGTACTGCAAGCGGGGCAGAAAGAAGCTGCTGTACATCTTCAAGCAGCCCTTCATGCGGCCCGTGCAGACCACACAAGAGGAAGATGGCTGCTCCTGCAGATTCCCCGAGGAAGAAGAAGGCGGCTGCGAGCTGAGAGTGAAGTTCTCTAGATCTGCCGACGCTCCTGCCTACCAGCAGGGACAGAATCAGCTGTACAACGAGCTGAATCTGGGGCGCAGAGAAGAGTACGACGTGCTGGATAAGAGAAGAGGCAGAGATCCCGAGATGGGCGGCAAGCCCCAGAGAAGAAAGAATCCCCAAGAGGGCCTGTATAATGAGCTGCAGAAAGACAAGATGGCCGAGGCCTACAGCGAGATCGGAATGAAGGGCGAACGCAGAAGAGGAAAGGGCCACGACGGACTGTATCAGGGCCTGAGCACAGCCACCAAGGATACCTATGATGCCCTGCACATGCAGGCCCTGCCACCTAGG

SEQ ID NO: 51 - protein, 1860 aa, synthetic construct
ATGGCCCTGCCTGTGACAGCTTTGCTGCTGCCTCTGGCTCTGCTGCTGCATGCTGCTAGACCTCAGATGCAGCTGGTGCAGTCTGGGGCTGAGGTGAAGAAGCCTGGGTCCTCGGTGAAGGTCTCCTGCAAGGCTTCTGGAGGCACCTTCAGCAGCTATGCTATCAGCTGGGTGCGACAGGCCCCTGGACAAGGGCTTGAGTGGATGGGAAGGATCATCCCTATCCTTGGTATAGCAAACTACGCACAGAAGTTCCAGGGCAGAGTCACGATTACCGCGGACAAATCCACGAGCACAGCCTACATGGAGCTGAGCAGCCTGAGATCTGAGGACACGGCCGTGTATTACTGTGCGAAACCGAGAGATGGCTACAATTTGGTTGCTTTTGATATCTGGGGCCAAGGGACGATGGTCACCGTCTCCTCAGGCCTCGGGGGCCTCGGAGGAGGAGGTAGTGGCGGAGGAGGCTCCGGTGGATCCAGCGGTGTGGGTTCCCAGCTCGTGCTGACTCAGCCGCCCTCAGTGTCTGGGGCCCCAGGGCAGAGGGTCACCATCTCCTGCACTGGGAGCAGCTCCAACATCGGGGCAGGTTATGATGTACACTGGTATCAGCAACTTCCAGGAGCAGCCCCCAAACTCCTCATCTATGGCGACATCAATCGGCCCTCAGGGGTCCCTGACCGATTCTCTGGCTCCAAGTCTGGCATCTCAGCCTCCCTGGCTATCACTGGGCTCCAGGCTGAGGACGAGGCTGATTATTACTGCCAGTCCTATGACAGCAGCCTGAGTGGGGGGGTGTTCGGCGGAGGGACCAAGCTGACCGTCCTAGGAGGCGGAGGTTCTGGCGGCGGAGGAAGTGGTGGCGGAGGCTCTAGCAGCGACAGCCCCAGAAATCTGGAAGTGACCAACGCCACACCTAACAGCCTGACCATCAGCTGGTACTACCCCTTCTGCGCCTTCTACTACCGGATCACCTATGGCGAGACAGGCGGCAACAGCCCTAGCCAAGAGTTCACCGTGCCTAGACCTAGCGACACCGCCACAATCTCTGGCCTGAAGCCAGGCCAGGACTACACCATCACAGTGTACGCCGTGACCTGCCTGGGCAGCTACAGCAGACCCATCAGCATCAACTACCGGACCGAGATCGACAAGCCCAGCCAAGACTACAAGGACGACGATGACAAGACCACCACACCAGCTCCACGGCCTCCAACACCAGCACCTACAATTGCCTCTCAGCCCCTGTCTCTGAGGCCAGAAGCTTGTAGACCTGCTGCAGGCGGAGCCGTGCATACCAGAGGACTGGATTTCGCCTGCGACATCTACATTTGGGCCCCTCTGGCTGGAACATGTGGCGTCCTGCTGCTGTCTCTCGTGATCACCCTGTACTGCAAGCGGGGCAGAAAGAAGCTGCTGTACATCTTCAAGCAGCCCTTCATGCGGCCCGTGCAGACCACACAAGAGGAAGATGGCTGCTCCTGCAGATTCCCCGAGGAAGAAGAAGGCGGCTGCGAGCTGAGAGTGAAGTTCTCTAGATCTGCCGACGCTCCTGCCTACCAGCAGGGACAGAATCAGCTGTACAACGAGCTGAATCTGGGGCGCAGAGAAGAGTACGACGTGCTGGATAAGAGAAGAGGCAGAGATCCCGAGATGGGCGGCAAGCCCCAGAGAAGAAAGAATCCCCAAGAGGGCCTGTATAATGAGCTGCAGAAAGACAAGATGGCCGAGGCCTACAGCGAGATCGGAATGAAGGGCGAACGCAGAAGAGGAAAGGGCCACGACGGACTGTATCAGGGCCTGAGCACAGCCACCAAGGATACCTATGATGCCCTGCACATGCAGGCCCTGCCACCTAGG

SEQ ID NO: 52 - protein, 1860 aa, synthetic construct
ATGGCCCTGCCTGTGACAGCTTTGCTGCTGCCTCTGGCTCTGCTGCTGCATGCTGCTAGACCTAGCAGCGACAGCCCCAGAAATCTGGAAGTGACCAACGCCACACCTAACAGCCTGACCATCAGCTGGTACTACCCCTTCTGCGCCTTCTACTACCGGATCACCTATGGCGAGACAGGCGGCAACAGCCCTAGCCAAGAGTTCACCGTGCCTAGACCTAGCGACACCGCCACAATCTCTGGCCTGAAGCCAGGCCAGGACTACACCATCACAGTGTACGCCGTGACCTGCCTGGGCAGCTACAGCAGACCCATCAGCATCAACTACCGGACCGAGATCGACAAGCCCAGCCAAGGAGGCGGAGGTTCTGGCGGCGGAGGAAGTGGTGGCGGAGGCTCTCAGATGCAGCTGGTGCAGTCTGGGGCTGAGGTGAAGAAGCCTGGGTCCTCGGTGAAGGTCTCCTGCAAGGCTTCTGGAGGCACCTTCAGCAGCTATGCTATCAGCTGGGTGCGACAGGCCCCTGGACAAGGGCTTGAGTGGATGGGAAGGATCATCCCTATCCTTGGTATAGCAAACTACGCACAGAAGTTCCAGGGCAGAGTCACGATTACCGCGGACAAATCCACGAGCACAGCCTACATGGAGCTGAGCAGCCTGAGATCTGAGGACACGGCCGTGTATTACTGTGCGAAACCGAGAGATGGCTACAATTTGGTTGCTTTTGATATCTGGGGCCAAGGGACGATGGTCACCGTCTCCTCAGGCCTCGGGGGCCTCGGAGGAGGAGGTAGTGGCGGAGGAGGCTCCGGTGGATCCAGCGGTGTGGGTTCCCAGCTCGTGCTGACTCAGCCGCCCTCAGTGTCTGGGGCCCCAGGGCAGAGGGTCACCATCTCCTGCACTGGGAGCAGCTCCAACATCGGGGCAGGTTATGATGTACACTGGTATCAGCAACTTCCAGGAGCAGCCCCCAAACTCCTCATCTATGGCGACATCAATCGGCCCTCAGGGGTCCCTGACCGATTCTCTGGCTCCAAGTCTGGCATCTCAGCCTCCCTGGCTATCACTGGGCTCCAGGCTGAGGACGAGGCTGATTATTACTGCCAGTCCTATGACAGCAGCCTGAGTGGGGGGGTGTTCGGCGGAGGGACCAAGCTGACCGTCCTAGACTACAAGGACGACGATGACAAGACCACCACACCAGCTCCACGGCCTCCAACACCAGCACCTACAATTGCCTCTCAGCCCCTGTCTCTGAGGCCAGAAGCTTGTAGACCTGCTGCAGGCGGAGCCGTGCATACCAGAGGACTGGATTTCGCCTGCGACATCTACATTTGGGCCCCTCTGGCTGGAACATGTGGCGTCCTGCTGCTGTCTCTCGTGATCACCCTGTACTGCAAGCGGGGCAGAAAGAAGCTGCTGTACATCTTCAAGCAGCCCTTCATGCGGCCCGTGCAGACCACACAAGAGGAAGATGGCTGCTCCTGCAGATTCCCCGAGGAAGAAGAAGGCGGCTGCGAGCTGAGAGTGAAGTTCTCTAGATCTGCCGACGCTCCTGCCTACCAGCAGGGACAGAATCAGCTGTACAACGAGCTGAATCTGGGGCGCAGAGAAGAGTACGACGTGCTGGATAAGAGAAGAGGCAGAGATCCCGAGATGGGCGGCAAGCCCCAGAGAAGAAAGAATCCCCAAGAGGGCCTGTATAATGAGCTGCAGAAAGACAAGATGGCCGAGGCCTACAGCGAGATCGGAATGAAGGGCGAACGCAGAAGAGGAAAGGGCCACGACGGACTGTATCAGGGCCTGAGCACAGCCACCAAGGATACCTATGATGCCCTGCACATGCAGGCCCTGCCACCTAGG

SEQ ID NO: 53 - protein, 619 aa, synthetic construct
MALPVTALLLPLALLLHAARPQMQLVQSGAEVKKPGSSVKVSCKASGGTFSSYAISWVRQAPGQGLEWMGRIIPILGIANYAQKFQGRVTITADKSTSTAYMELSSLRSEDTAVYYCAKPRDGYNLVAFDIWGQGTMVTVSSGLGGLGGGGSGGGGSGGSSGVGSQLVLTQPPSVSGAPGQRVTISCTGSSSNIGAGYDVHWYQQLPGAAPKLLIYGDINRPSGVPDRFSGSKSGISASLAITGLQAEDEADYYCQSYDSSLSGGVFGGGTKLTVLGGGGSGGGGSGGGGSSSDSPRNLEVTNATPNSLTISWYYPFCAFYYRITYGETGGNSPSQEFTVPRPSDTATISGLKPGQDYTITVYAVTCLGSYSRPISINYRTEIDKPSQDYKDDDDKTTTPAPRPPTPAPTIASQPLSLRPEACRPAAGGAVHTRGLDFACDIYIWAPLAGTCGVLLLSLVITLYCRSKRSRLLHSDYMNMTPRRPGPTRKHYQPYAPPRDFAAYRSRVKFSRSADAPAYQQGQNQLYNELNLGRREEYDVLDKRRGRDPEMGGKPQRRKNPQEGLYNELQKDKMAEAYSEIGMKGERRRGKGHDGLYQGLSTATKDTYDALHMQALPPR

SEQ ID NO: 54 - protein, 619 aa, synthetic construct
MALPVTALLLPLALLLHAARPSSDSPRNLEVTNATPNSLTISWYYPFCAFYYRITYGETGGNSPSQEFTVPRPSDTATISGLKPGQDYTITVYAVTCLGSYSRPISINYRTEIDKPSQGGGGSGGGGSGGGGSQMQLVQSGAEVKKPGSSVKVSCKASGGTFSSYAISWVRQAPGQGLEWMGRIIPILGIANYAQKFQGRVTITADKSTSTAYMELSSLRSEDTAVYYCAKPRDGYNLVAFDIWGQGTMVTVSSGLGGLGGGGSGGGGSGGSSGVGSQLVLTQPPSVSGAPGQRVTISCTGSSSNIGAGYDVHWYQQLPGAAPKLLIYGDINRPSGVPDRFSGSKSGISASLAITGLQAEDEADYYCQSYDSSLSGGVFGGGTKLTVLDYKDDDDKTTTPAPRPPTPAPTIASQPLSLRPEACRPAAGGAVHTRGLDFACDIYIWAPLAGTCGVLLLSLVITLYCRSKRSRLLHSDYMNMTPRRPGPTRKHYQPYAPPRDFAAYRSRVKFSRSADAPAYQQGQNQLYNELNLGRREEYDVLDKRRGRDPEMGGKPQRRKNPQEGLYNELQKDKMAEAYSEIGMKGERRRGKGHDGLYQGLSTATKDTYDALHMQALPPR

SEQ ID NO: 55 - protein, 341 aa, synthetic construct
MALPVTALLLPLALLLHAARPSSDSPRNLEVTNATPNSLTISWYYPFCAFYYRITYGETGGNSPSQEFTVPRPSDTATISGLKPGQDYTITVYAVTCLGSYSRPISINYRTEIDKPSQTTTPAPRPPTPAPTIASQPLSLRPEACRPAAGGAVHTRGLDFACDIYIWAPLAGTCGVLLLSLVITLYCRSKRSRLLHSDYMNMTPRRPGPTRKHYQPYAPPRDFAAYRSRVKFSRSADAPAYQQGQNQLYNELNLGRREEYDVLDKRRGRDPEMGGKPQRRKNPQEGLYNELQKDKMAEAYSEIGMKGERRRGKGHDGLYQGLSTATKDTYDALHMQALPPR

SEQ ID NO: 56 - protein, 342 aa, synthetic construct
MALPVTALLLPLALLLHAARPSSDSPRNLEVTNATPNSLTISWYYPFCAFYYRITYGETGGNSPSQEFTVPRPSDTATISGLKPGQDYTITVYAVTCLGSYSRPISINYRTEIDKPSQTTTPAPRPPTPAPTIASQPLSLRPEACRPAAGGAVHTRGLDFACDIYIWAPLAGTCGVLLLSLVITLYCKRGRKKLLYIFKQPFMRPVQTTQEEDGCSCRFPEEEEGGCELRVKFSRSADAPAYQQGQNQLYNELNLGRREEYDVLDKRRGRDPEMGGKPQRRKNPQEGLYNELQKDKMAEAYSEIGMKGERRRGKGHDGLYQGLSTATKDTYDALHMQALPPR

SEQ ID NO: 57 - protein, 620 aa, synthetic construct
MALPVTALLLPLALLLHAARPQMQLVQSGAEVKKPGSSVKVSCKASGGTFSSYAISWVRQAPGQGLEWMGRIIPILGIANYAQKFQGRVTITADKSTSTAYMELSSLRSEDTAVYYCAKPRDGYNLVAFDIWGQGTMVTVSSGLGGLGGGGSGGGGSGGSSGVGSQLVLTQPPSVSGAPGQRVTISCTGSSSNIGAGYDVHWYQQLPGAAPKLLIYGDINRPSGVPDRFSGSKSGISASLAITGLQAEDEADYYCQSYDSSLSGGVFGGGTKLTVLGGGGSGGGGSGGGGSSSDSPRNLEVTNATPNSLTISWYYPFCAFYYRITYGETGGNSPSQEFTVPRPSDTATISGLKPGQDYTITVYAVTCLGSYSRPISINYRTEIDKPSQDYKDDDDKTTTPAPRPPTPAPTIASQPLSLRPEACRPAAGGAVHTRGLDFACDIYIWAPLAGTCGVLLLSLVITLYCKRGRKKLLYIFKQPFMRPVQTTQEEDGCSCRFPEEEEGGCELRVKFSRSADAPAYQQGQNQLYNELNLGRREEYDVLDKRRGRDPEMGGKPQRRKNPQEGLYNELQKDKMAEAYSEIGMKGERRRGKGHDGLYQGLSTATKDTYDALHMQALPPR

SEQ ID NO: 58 - protein, 620 aa, synthetic construct
MALPVTALLLPLALLLHAARPSSDSPRNLEVTNATPNSLTISWYYPFCAFYYRITYGETGGNSPSQEFTVPRPSDTATISGLKPGQDYTITVYAVTCLGSYSRPISINYRTEIDKPSQGGGGSGGGGSGGGGSQMQLVQSGAEVKKPGSSVKVSCKASGGTFSSYAISWVRQAPGQGLEWMGRIIPILGIANYAQKFQGRVTITADKSTSTAYMELSSLRSEDTAVYYCAKPRDGYNLVAFDIWGQGTMVTVSSGLGGLGGGGSGGGGSGGSSGVGSQLVLTQPPSVSGAPGQRVTISCTGSSSNIGAGYDVHWYQQLPGAAPKLLIYGDINRPSGVPDRFSGSKSGISASLAITGLQAEDEADYYCQSYDSSLSGGVFGGGTKLTVLDYKDDDDKTTTPAPRPPTPAPTIASQPLSLRPEACRPAAGGAVHTRGLDFACDIYIWAPLAGTCGVLLLSLVITLYCKRGRKKLLYIFKQPFMRPVQTTQEEDGCSCRFPEEEEGGCELRVKFSRSADAPAYQQGQNQLYNELNLGRREEYDVLDKRRGRDPEMGGKPQRRKNPQEGLYNELQKDKMAEAYSEIGMKGERRRGKGHDGLYQGLSTATKDTYDALHMQALPPR